European Patent Specification EP 3 230 312 B1, published January 24, 2024. Title: A method for producing a recombinant allotype-specific rabbit monoclonal antibody. Applicant: Abcam plc. The sequence listing filed with the application follows.

SEQUENCE LISTING (22 sequences)

SEQ ID NO: 1 - DNA, 20 bp, Artificial Sequence
  source 1..20: /organism="Artificial Sequence" /note="3’ end of b4 kappa light chain forward primer " /mol_type="unassigned DNA"
atggacacgagggcccccac

SEQ ID NO: 2 - DNA, 10 bp, Artificial Sequence
  source 1..10: /organism="Artificial Sequence" /note="3’ end of b4 kappa light chain reverse primer " /mol_type="unassigned DNA"
  misc_feature 10: /note="a is a or ac or acc or accc"
ctaacagtca

SEQ ID NO: 3 - DNA, 23 bp, Artificial Sequence
  source 1..23: /organism="Artificial Sequence" /note="3’ end of b4 heavy chain forward primer" /mol_type="unassigned DNA"
atggagactgggctgcgctggct

SEQ ID NO: 4 - DNA, 18 bp, Artificial Sequence
  source 1..18: /organism="Artificial Sequence" /note="3’ end of b4 heavy chain reverse primer" /mol_type="unassigned DNA"
caggcagcccagggtcac

SEQ ID NO: 5 - DNA, 12 bp, Artificial Sequence
  source 1..12: /organism="Artificial Sequence" /note="3’ end of b4 kappa light chain reverse primer" /mol_type="unassigned DNA"
ctaacagtcacc

SEQ ID NO: 6 - DNA, 41 bp, Artificial Sequence
  source 1..41: /organism="Artificial Sequence" /note="3’ end of b4 kappa light chain forward primer" /mol_type="unassigned DNA"
cgcaagcttgtacccttcaccatggacacgagggcccccac

SEQ ID NO: 7 - DNA, 30 bp, Artificial Sequence
  source 1..30: /organism="Artificial Sequence" /note="3’ end of b4 kappa light chain reverse primer" /mol_type="unassigned DNA"
  misc_feature 16: /note="r is g or a"
cgcgcggccgctctcrctctaacagtcacc

SEQ ID NO: 8 - DNA, 44 bp, Artificial Sequence
  source 1..44: /organism="Artificial Sequence" /note="3’ end of heavy chain forward primer" /mol_type="unassigned DNA"
cggaagcttgtacccttcaccatggagactgggctgcgctggct

SEQ ID NO: 9 - DNA, 35 bp, Artificial Sequence
  source 1..35: /organism="Artificial Sequence" /note="3’ end of heavy chain reverse primer" /mol_type="unassigned DNA"
gggaggtaccctttgaccaggcagcccagggtcac

SEQ ID NO: 10 - DNA, 68 bp, Artificial Sequence
  source 1..68: /organism="Artificial Sequence" /note="cDNA of 5’ end of an exemplary kappa light chain" /mol_type="unassigned DNA"
cagtgcaggcaggacccagcatggacacgagggcccccactcagctgctggggctcctgctgctctgg

SEQ ID NO: 11 - DNA, 10 bp, Artificial Sequence
  source 1..10: /organism="Artificial Sequence" /note="3’ end of b4 kappa light chain reverse primer" /mol_type="unassigned DNA"
  misc_feature 4: /note="r is g or a"
  misc_feature 10: /note="a is a or ac or acc or accc"
ctarcagtca

SEQ ID NO: 12 - DNA, 12 bp, Artificial Sequence
  source 1..12: /organism="Artificial Sequence" /note="3’ end of b4 kappa light chain reverse primer" /mol_type="unassigned DNA"
  misc_feature 4: /note="r is g or a"
ctarcagtcacc

SEQ ID NO: 13 - protein, 16 aa, Artificial Sequence
  Encoded amino acid sequence of SEQ ID No: 10
MDTRAPTQLLGLLLLW

SEQ ID NO: 14 - DNA, 58 bp, Artificial Sequence
  source 1..58: /organism="Artificial Sequence" /note="cDNA of 3’ end of an exemplary kappa light chain" /mol_type="unassigned DNA"
ggcacgacctcagtcgtccagagcttcaataggggtgactgttagagcgagacgcctg

SEQ ID NO: 15 - protein, 14 aa, Artificial Sequence
  Encoded amino acid sequence of SEQ ID No: 14
GTTSVVQSFNRGDC

SEQ ID NO: 16 - DNA, 12 bp, Artificial Sequence
  source 1..12: /organism="Artificial Sequence" /note="3’ end of b4 kappa light chain reverse primer" /mol_type="unassigned DNA"
ctaacagtcaca

SEQ ID NO: 17 - DNA, 12 bp, Artificial Sequence
  source 1..12: /organism="Artificial Sequence" /note="3’ end of b4 kappa light chain reverse primer" /mol_type="unassigned DNA"
ctagcagtcaca

SEQ ID NO: 18 - DNA, 12 bp, Artificial Sequence
  source 1..12: /organism="Artificial Sequence" /note="3’ end of b4 kappa light chain reverse primer" /mol_type="unassigned DNA"
ctaacagtcacc

SEQ ID NO: 19 - DNA, 12 bp, Artificial Sequence
  source 1..12: /organism="Artificial Sequence" /note="3’ end of b4 kappa light chain reverse primer" /mol_type="unassigned DNA"
ctagcagtcacc

SEQ ID NO: 20 - DNA, 12 bp, Artificial Sequence
  source 1..12: /organism="Artificial Sequence" /note="3’ end of b4 kappa light chain reverse primer" /mol_type="unassigned DNA"
ctagcagtcacc

SEQ ID NO: 21 - DNA, 13 bp, Artificial Sequence
  source 1..13: /organism="Artificial Sequence" /note="3’ end of b4 kappa light chain reverse primer" /mol_type="unassigned DNA"
ctaacagtcaccc

SEQ ID NO: 22 - DNA, 13 bp, Artificial Sequence
  source 1..13: /organism="Artificial Sequence" /note="3’ end of b4 kappa light chain reverse primer" /mol_type="unassigned DNA"
ctagcagtcaccc